European Patent Application EP 4 269 436 A1, published November 1, 2023. Title: CLAUDIN18.2 CHIMERIC ANTIGEN RECEPTOR AND USE THEREOF. Applicant: Innovent Biologics (Suzhou) Co., Ltd. The sequence listing filed with the application follows.

SEQUENCE LISTING (89 sequences)

SEQ ID NO: 1 - protein, 10 aa, Artificial
  Synthetic polypeptide/peptide
GFSFSDYGMH

SEQ ID NO: 2 - protein, 17 aa, Artificial
  Synthetic polypeptide/peptide
YINSGSRTLYYADTVKG

SEQ ID NO: 3 - protein, 10 aa, Artificial
  Synthetic polypeptide/peptide
NAYYGNAMDY

SEQ ID NO: 4 - protein, 119 aa, Artificial
  Synthetic polypeptide/peptide
EVQLVESGGGLVQPGGSLRLSCAASGFSFSDYGMHWVRQAPGKGLEWVSYINSGSRTLYYADTVKGRFTISRDNAKNSLYLQMNSLRDEDTAVYYCARNAYYGNAMDYWGQGTLVTVSS

SEQ ID NO: 5 - protein, 330 aa, Artificial
  Synthetic polypeptide/peptide
ASTKGPSVFPLAPSSKSTSGGTAALGCLVKDYFPEPVTVSWNSGALTSGVHTFPAVLQSSGLYSLSSVVTVPSSSLGTQTYICNVNHKPSNTKVDKKAEPKSCDKTHTCPPCPAPELLGGPSVFLFPPKPKDTLMISRTPEVTCVVVDVSHEDPEVKFNWYVDGVEVHNAKTKPREEQYNSTYRVVSVLTVLHQDWLNGKEYKCKVSNKALPAPIEKTISKAKGQPREPQVYTLPPSRDELTKNQVSLTCLVKGFYPSDIAVEWESNGQPENNYKTTPPVLDSDGSFFLYSKLTVDKSRWQQGNVFSCSVMHEALHNHYTQKSLSLSPGK

SEQ ID NO: 6 - protein, 17 aa, Artificial
  Synthetic polypeptide/peptide
KSSQSLLNSGNQRNYLT

SEQ ID NO: 7 - protein, 7 aa, Artificial
  Synthetic polypeptide/peptide
WSSTRGS

SEQ ID NO: 8 - protein, 9 aa, Artificial
  Synthetic polypeptide/peptide
QNVYYYPFT

SEQ ID NO: 9 - protein, 113 aa, Artificial
  Synthetic polypeptide/peptide
DIVMTQSPDSLAVSLGERATINCKSSQSLLNSGNQRNYLTWYQQKPGQPPKLLIYWSSTRGSGVPDRFSGSGSGTDFTLTISSLQAEDVAVYYCQNVYYYPFTFGQGTRLEIK

SEQ ID NO: 10 - protein, 107 aa, Artificial [sequence omitted]

SEQ ID NO: 11 - protein, 247 aa, Artificial
  Synthetic polypeptide/peptide
EVQLVESGGGLVQPGGSLRLSCAASGFSFSDYGMHWVRQAPGKGLEWVSYINSGSRTLYYADTVKGRFTISRDNAKNSLYLQMNSLRDEDTAVYYCARNAYYGNAMDYWGQGTLVTVSSGGGGSGGGGSGGGGSDIVMTQSPDSLAVSLGERATINCKSSQSLLNSGNQRNYLTWYQQKPGQPPKLLIYWSSTRGSGVPDRFSGSGSGTDFTLTISSLQAEDVAVYYCQNVYYYPFTFGQGTRLEIK

SEQ ID NO: 12 - protein, 15 aa, Artificial
  Synthetic polypeptide/peptide
GGGGSGGGGSGGGGS

SEQ ID NO: 13 - protein, 10 aa, Artificial
  Synthetic polypeptide/peptide
GFSLTDYGVS

SEQ ID NO: 14 - protein, 16 aa, Artificial
  Synthetic polypeptide/peptide
VMWGGGNTYYNSALKS

SEQ ID NO: 15 - protein, 10 aa, Artificial
  Synthetic polypeptide/peptide
QRYGGNAMDY

SEQ ID NO: 16 - protein, 118 aa, Artificial
  Synthetic polypeptide/peptide
QVQLQESGPGLVKPSETLSLTCTVSGFSLTDYGVSWIRQPPGKGLEWIGVMWGGGNTYYNSALKSRVTISVDTSKNQFSLKLSSVTAADTAVYYCARQRYGGNAMDYWGQGTLVTVSS

SEQ ID NO: 17 - protein, 7 aa, Artificial
  Synthetic polypeptide/peptide
WASTRES

SEQ ID NO: 18 - protein, 9 aa, Artificial
  Synthetic polypeptide/peptide
QNSYFYPFT

SEQ ID NO: 19 - protein, 113 aa, Artificial
  Synthetic polypeptide/peptide
DIVMTQSPDSLAVSLGERATINCKSSQSLLNSGNQRNYLTWYQQKPGQPPKLLIYWASTRESGVPDRFSGSGSGTDFTLTISSLQAEDVAVYYCQNSYFYPFTFGGGTKVEIK

SEQ ID NO: 20 - protein, 246 aa, Artificial
  Synthetic polypeptide/peptide
QVQLQESGPGLVKPSETLSLTCTVSGFSLTDYGVSWIRQPPGKGLEWIGVMWGGGNTYYNSALKSRVTISVDTSKNQFSLKLSSVTAADTAVYYCARQRYGGNAMDYWGQGTLVTVSSGGGGSGGGGSGGGGSDIVMTQSPDSLAVSLGERATINCKSSQSLLNSGNQRNYLTWYQQKPGQPPKLLIYWASTRESGVPDRFSGSGSGTDFTLTISSLQAEDVAVYYCQNSYFYPFTFGGGTKVEIK

SEQ ID NO: 21 - protein, 10 aa, Artificial
  Synthetic polypeptide/peptide
GFSLNSYGVG

SEQ ID NO: 22 - protein, 16 aa, Artificial
  Synthetic polypeptide/peptide
VIWGDVSTNYHSVLIS

SEQ ID NO: 23 - protein, 9 aa, Artificial
  Synthetic polypeptide/peptide
ITRGNAMDY

SEQ ID NO: 24 - protein, 117 aa, Artificial
  Synthetic polypeptide/peptide
QVQLQESGPGLVKPSETLSLTCTVSGFSLNSYGVGWIRQPPGKGLEWIGVIWGDVSTNYHSVLISRVTISKDTSKNQVSLKLSSVTAADTAVYYCARITRGNAMDYWGQGTLVTVSS

SEQ ID NO: 25 - protein, 7 aa, Artificial
  Synthetic polypeptide/peptide
WASTRKS

SEQ ID NO: 26 - protein, 9 aa, Artificial
  Synthetic polypeptide/peptide
QNNYLFPLT

SEQ ID NO: 27 - protein, 113 aa, Artificial
  Synthetic polypeptide/peptide
DIVMTQSPDSLAVSLGERATINCKSSQSLLNSGNQRNYLTWYQQKPGQPPKLLIYWASTRKSGVPDRFSGSGSGTDFTLTISSLQAEDVAVYYCQNNYLFPLTFGGGTKVEIK

SEQ ID NO: 28 - protein, 245 aa, Artificial
  Synthetic polypeptide/peptide
QVQLQESGPGLVKPSETLSLTCTVSGFSLNSYGVGWIRQPPGKGLEWIGVIWGDGSTNYHSVLISRVTISVDTSKNQFSLKLSSVTAADTAVYYCARITRGNAMDYWGQGTLVTVSSGGGGSGGGGSGGGGSDIVMTQSPDSLAVSLGERATINCKSSQSLLNSGNQRNYLTWYQQKPGQPPKLLIYWASTRKSGVPDRFSGSGSGTDFTLTISSLQAEDVAVYYCQNNYLFPLTFGGGTKVEIK

SEQ ID NO: 29 - protein, 10 aa, Artificial
  Synthetic polypeptide/peptide
GFTFSDYGMA

SEQ ID NO: 30 - protein, 17 aa, Artificial
  Synthetic polypeptide/peptide
FINNLAYSIYYVDTVTG

SEQ ID NO: 31 - protein, 9 aa, Artificial
  Synthetic polypeptide/peptide
FTTGNVMDY

SEQ ID NO: 32 - protein, 118 aa, Artificial
  Synthetic polypeptide/peptide
EVQLVESGGGLVQPGGSLRLSCAASGFTFSDYGMAWVRQAPGKGLEWVAFINNLAYSIYYVDTVTGRFTISRDNAKNSLYLQMNSLRAEDTAVYYCARFTTGNVMDYWGQGTLVTVSS

SEQ ID NO: 33 - protein, 17 aa, Artificial
  Synthetic polypeptide/peptide
KSSQSLLQGGNQKNYLT

SEQ ID NO: 34 - protein, 7 aa, Artificial
  Synthetic polypeptide/peptide
WSSTRES

SEQ ID NO: 35 - protein, 9 aa, Artificial
  Synthetic polypeptide/peptide
QNSYSYPLT

SEQ ID NO: 36 - protein, 113 aa, Artificial
  Synthetic polypeptide/peptide
DIVMTQSPDSLAVSLGERATINCKSSQSLLQGGNQKNYLTWYQQKPGQPPKLLIYWSSTRESGVPDRFSGSGSGTDFTLTISSLQAEDVAVYYCQNSYSYPLTFGGGTKVEIK

SEQ ID NO: 37 - protein, 246 aa, Artificial
  Synthetic polypeptide/peptide
EVQLVESGGGLVQPGGSLRLSCAASGFTFSDYGMAWVRQAPGKGLEWVAFINNLAYSIYYVDTVTGRFTISRDNAKNSLYLQMNSLRAEDTAVYYCARFTTGNVMDYWGQGTLVTVSSGGGGSGGGGSGGGGSDIVMTQSPDSLAVSLGERATINCKSSQSLLNGGNQKNYLTWYQQKPGQPPKLLIYWSSTRESGVPDRFSGSGSGTDFTLTISSLQAEDVAVYYCQNSYSYPLTFGGGTKVEIK

SEQ ID NO: 38 - protein, 10 aa, Artificial
  Synthetic polypeptide/peptide
GYSFSSYNIH

SEQ ID NO: 39 - protein, 17 aa, Artificial
  Synthetic polypeptide/peptide
YIAPFQGDSRYNQKFKG

SEQ ID NO: 40 - protein, 9 aa, Artificial
  Synthetic polypeptide/peptide
LNRGNSLDY

SEQ ID NO: 41 - protein, 118 aa, Artificial
  Synthetic polypeptide/peptide
QVQLVQSGAEVKKPGSSVKVSCKASGYSFSSYNIHWVRQAPGQGLEWMGYIAPFQGDSRYNQKFKGRVTITADKSTSTAYMELSSLRSEDTAVYYCARLNRGNSLDYWGQGTLVTVSS

SEQ ID NO: 42 - protein, 17 aa, Artificial
  Synthetic polypeptide/peptide
KSSQSLFNSGNQRNYLT

SEQ ID NO: 43 - protein, 9 aa, Artificial
  Synthetic polypeptide/peptide
QNNYIYPLT

SEQ ID NO: 44 - protein, 113 aa, Artificial
  Synthetic polypeptide/peptide
DIVMTQSPDSLAVSLGERATINCKSSQSLFNSGNQRNYLTWYQQKPGQPPKLLIYWASTRESGVPDRFSGSGSGTDFTLTISSLQAEDVAVYYCQNNYIYPLTFGGGTKVEIK

SEQ ID NO: 45 - protein, 246 aa, Artificial
  Synthetic polypeptide/peptide
QVQLVQSGAEVKKPGSSVKVSCKASGYSFSSYNIHWVRQAPGQGLEWMGYIAPFQGDSRYNQKFKGRVTITADKSTSTAYMELSSLRSEDTAVYYCARLNRGNSLDYWGQGTLVTVSSGGGGSGGGGSGGGGSDIVMTQSPDSLAVSLGERATINCKSSQSLFNSGNQRNYLTWYQQKPGQPPKLLIYWASTRESGVPDRFSGSGSGTDFTLTISSLQAEDVAVYYCQNNYIYPLTFGGGTKVEIK

SEQ ID NO: 46 - protein, 11 aa, Artificial
  Synthetic polypeptide/peptide
GYSITSGYGWN

SEQ ID NO: 47 - protein, 16 aa, Artificial
  Synthetic polypeptide/peptide
YIHFSGSTNYNPSLKS

SEQ ID NO: 48 - protein, 9 aa, Artificial
  Synthetic polypeptide/peptide
SGKGNAMDY

SEQ ID NO: 49 - protein, 118 aa, Artificial
  Synthetic polypeptide/peptide
QVQLQESGPGLVKPSETLSLTCTVSGYSITSGYGWNWIRQPPGKGLEWIGYIHFSGSTNYNPSLKSRVTISVDTSKNQFSLKLSSVTAADTAVYYCARSGKGNAMDYWGQGTLVTVSS

SEQ ID NO: 50 - protein, 17 aa, Artificial
  Synthetic polypeptide/peptide
KSSQSLLNSGNQKNYLT

SEQ ID NO: 51 - protein, 9 aa, Artificial
  Synthetic polypeptide/peptide
QNDYYFPFT

SEQ ID NO: 52 - protein, 113 aa, Artificial
  Synthetic polypeptide/peptide
DIVMTQSPDSLAVSLGERATINCKSSQSLLNSGNQKNYLTWYQQKPGQPPKLLIYWASTRESGVPDRFSGSGSGTDFTLTISSLQAEDVAVYYCQNDYYFPFTFGGGTKVEIK

SEQ ID NO: 53 - protein, 246 aa, Artificial
  Synthetic polypeptide/peptide
QVQLQESGPGLVKPSETLSLTCTVSGYSITSGYGWNWIRQPPGKGLEWIGYIHFSGSTNYNPSLKSRVTISVDTSKNQFSLKLSSVTAADTAVYYCARSGKGNAMDYWGQGTLVTVSSGGGGSGGGGSGGGGSDIVMTQSPDSLAVSLGERATINCKSSQSLLNSGNQKNYLTWYQQKPGQPPKLLIYWASTRESGVPDRFSGSGSGTDFTLTISSLQAEDVAVYYCQNDYYFPFTFGGGTKVEIK

SEQ ID NO: 54 - protein, 10 aa, Artificial
  Synthetic polypeptide/peptide
GYSFTTYWMH

SEQ ID NO: 55 - protein, 17 aa, Artificial
  Synthetic polypeptide/peptide
LIDPSDSETRLNQKFKD

SEQ ID NO: 56 - protein, 6 aa, Artificial
  Synthetic polypeptide/peptide
NRWLLG

SEQ ID NO: 57 - protein, 115 aa, Artificial
  Synthetic polypeptide/peptide
QVQLVQSGAEVKKPGASVKVSCKASGYSFTTYWMHWVRQAPGQGLEWMGLIDPSDSETRLNQKFKDRVTMTVDTSTSTVYMELSSLRSEDTAVYYCASNRWLLGWGQGTLVTVSS

SEQ ID NO: 58 - protein, 9 aa, Artificial
  Synthetic polypeptide/peptide
QNDYSYPLT

SEQ ID NO: 59 - protein, 113 aa, Artificial
  Synthetic polypeptide/peptide
DIVMTQSPDSLAVSLGERATINCKSSQSLLNSGNQKNYLTWYQQKPGQPPKLLIYWASTRESGVPDRFSGSGSGTDFTLTISSLQAEDVAVYYCQNDYSYPLTFGQGTKLEIK

SEQ ID NO: 60 - protein, 243 aa, Artificial
  Synthetic polypeptide/peptide
QVQLVQSGAEVKKPGASVKVSCKASGYSFTTYWMHWVRQAPGQGLEWMGLIDPSDSETRLNQKFKDRVTMTVDTSTSTVYMELSSLRSEDTAVYYCASNRWLLGWGQGTLVTVSSGGGGSGGGGSGGGGSDIVMTQSPDSLAVSLGERATINCKSSQSLLNSGNQKNYLTWYQQKPGQPPKLLIYWASTRESGVPDRFSGSGSGTDFTLTISSLQAEDVAVYYCQNDYSYPLTFGQGTKLEIK

SEQ ID NO: 61 - protein, 10 aa, Artificial
  Synthetic polypeptide/peptide
GYTFTKYIIQ

SEQ ID NO: 62 - protein, 17 aa, Artificial
  Synthetic polypeptide/peptide
YINPYNDDTKYNEKFKG

SEQ ID NO: 63 - protein, 9 aa, Artificial
  Synthetic polypeptide/peptide
TYYGNSFPN

SEQ ID NO: 64 - protein, 118 aa, Artificial
  Synthetic polypeptide/peptide
QVQLVQSGAEVKKPGASVKVSCKASGYTFTKYIIQWVRQAPGQRLEWMGYINPYNDDTKYNEKFKGRVTITRDTSASTAYMELSSLRSEDMAVYYCARTYYGNSFPNWGQGTLVTVSS

SEQ ID NO: 65 - protein, 9 aa, Artificial
  Synthetic polypeptide/peptide
QNDYSFPFT

SEQ ID NO: 66 - protein, 113 aa, Artificial
  Synthetic polypeptide/peptide
DIVMTQSPDSLAVSLGERATINCKSSQSLLNSGNQKNYLTWYQQKPGQPPKLLIYWASTRESGVPDRFSGSGSGTDFTLTISSLQAEDVAVYYCQNDYSFPFTFGGGTKVEIK

SEQ ID NO: 67 - protein, 246 aa, Artificial
  Synthetic polypeptide/peptide
QVQLVQSGAEVKKPGASVKVSCKASGYTFTKYIIQWVRQAPGQRLEWMGYINPYNDDTKYNEKFKGRVTITRDTSASTAYMELSSLRSEDMAVYYCARTYYGNSFPNWGQGTLVTVSSGGGGSGGGGSGGGGSDIVMTQSPDSLAVSLGERATINCKSSQSLLNSGNQKNYLTWYQQKPGQPPKLLIYWASTRESGVPDRFSGSGSGTDFTLTISSLQAEDVAVYYCQNDYSFPFTFGGGTKVEIK

SEQ ID NO: 68 - protein, 10 aa, Artificial
  Synthetic polypeptide/peptide
GFTFSSYVMS

SEQ ID NO: 69 - protein, 17 aa, Artificial
  Synthetic polypeptide/peptide
TISHSGGSTYYADSVKG

SEQ ID NO: 70 - protein, 13 aa, Artificial
  Synthetic polypeptide/peptide
DAPYYDILTGYRY

SEQ ID NO: 71 - protein, 122 aa, Artificial
  Synthetic polypeptide/peptide
EVQLLDSGGGLVQPGGSLRLSCAASGFTFSSYVMSWVRQAPGKGLNWVSTISHSGGSTYYADSVKGRFTISRDNSKNTLYLQMNSLRAEDTAVYYCAIDAPYYDILTGYRYWGQGTLVTVSS

SEQ ID NO: 72 - protein, 11 aa, Artificial
  Synthetic polypeptide/peptide
RASQSISSWLA

SEQ ID NO: 73 - protein, 7 aa, Artificial
  Synthetic polypeptide/peptide
KASSLES

SEQ ID NO: 74 - protein, 9 aa, Artificial
  Synthetic polypeptide/peptide
QQYNSYSYT

SEQ ID NO: 75 - protein, 107 aa, Artificial
  Synthetic polypeptide/peptide
DIQMTQSPSTLSASVGDRVTITCRASQSISSWLAWYQQKPGKAPKLLIYKASSLESGVPSRFSGSGSGTEFTLTISSLQPDDFATYYCQQYNSYSYTFGQGTKLEIK

SEQ ID NO: 76 - protein, 244 aa, Artificial
  Synthetic polypeptide/peptide
EVQLLDSGGGLVQPGGSLRLSCAASGFTFSSYVMSWVRQAPGKGLNWVSTISHSGGSTYYADSVKGRFTISRDNSKNTLYLQMNSLRAEDTAVYYCAIDAPYYDILTGYRYWGQGTLVTVSSGGGGSGGGGSGGGGSDIQMTQSPSTLSASVGDRVTITCRASQSISSWLAWYQQKPGKAPKLLIYKASSLESGVPSRFSGSGSGTEFTLTISSLQPDDFATYYCQQYNSYSYTFGQGTKLEIK

SEQ ID NO: 77 - protein, 10 aa, Artificial
  Synthetic polypeptide/peptide
GCCACCATGG

SEQ ID NO: 78 - protein, 21 aa, Artificial
  Synthetic polypeptide/peptide
MALPVTALLLPLALLLHAARP

SEQ ID NO: 79 - protein, 45 aa, Artificial
  Synthetic polypeptide/peptide
TTTPAPRPPTPAPTIASQPLSLRPEACRPAAGGAVHTRGLDFACD

SEQ ID NO: 80 - protein, 27 aa, Artificial
  Synthetic polypeptide/peptide
FWVLVVVGGVLACYSLLVTVAFIIFWV

SEQ ID NO: 81 - protein, 41 aa, Artificial
  Synthetic polypeptide/peptide
RSKRSRLLHSDYMNMTPRRPGPTRKHYQPYAPPRDFAAYRS

SEQ ID NO: 82 - protein, 112 aa, Artificial
  Synthetic polypeptide/peptide
RVKFSRSADAPAYQQGQNQLYNELNLGRREEYDVLDKRRGRDPEMGGKPRRKNPQEGLYNELQKDKMAEAYSEIGMKGERRRGKGHDGLYQGLSTATKDTYDALHMQALPPR

SEQ ID NO: 83 - protein, 18 aa, Artificial
  Synthetic polypeptide/peptide
EGRGSLLTCGDVEENPGP

SEQ ID NO: 84 - protein, 198 aa, Artificial
  Synthetic polypeptide/peptide
MVSKGEELFTGVVPILVELDGDVNGHKFSVSGEGEGDATYGKLTLKFICTTGKLPVPWPTLVTTLTYGVQCFSRYPDHMKQHDFFKSAMPEGYVQERTIFFKDDGNYKTRAEVKFEGDTLVNRIELKGIDFKEDGNILGHKLEYNYNSHNVYIMADKQKNGIKVNFKIRHNIEDGSVQLADHYQQNTPIGDGPVLLPD

SEQ ID NO: 85 - protein, 257 aa, Artificial
  Synthetic polypeptide/peptide
EGRGSLLTCGDVEENPGPMVSKGEELFTGVVPILVELDGDVNGHKFSVSGEGEGDATYGKLTLKFICTTGKLPVPWPTLVTTLTYGVQCFSRYPDHMKQHDFFKSAMPEGYVQERTIFFKDDGNYKTRAEVKFEGDTLVNRIELKGIDFKEDGNILGHKLEYNYNSHNVYIMADKQKNGIKVNFKIRHNIEDGSVQLADHYQQNTPIGDGPVLLPDNHYLSTQSALSKDPNEKRDHMVLLEFVTAAGITLGMDELYK

SEQ ID NO: 86 - protein, 24 aa, Artificial
  Synthetic polypeptide/peptide
IYIWAPLAGTCGVLLLSLVITLYC

SEQ ID NO: 87 - protein, 42 aa, Artificial
  Synthetic polypeptide/peptide
KRGRKKLLYIFKQPFMRPVQTTQEEDGCSCRFPEEEEGGCEL

SEQ ID NO: 88 - protein, 247 aa, Artificial
  Synthetic polypeptide/peptide
QVQLQESGPGLIKPSQTLSLTCTVSGGSISSGYNWHWIRQPPGKGLEWIGYIHYTGSTNYNPALRSRVTISVDTSKNQFSLKLSSVTAADTAIYYCARIYNGNSFPYWGQGTTVTVSSGGGGSGGGGSGGGGSDIVMTQSPDSLAVSLGERATINCKSSQSLFNSGNQKNYLTWYQQKPGQPPKLLIYWASTRESGVPDRFSGSGSGTDFTLTISSLQAEDVAVYYCQNAYSFPYTFGGGTKLEIKR

SEQ ID NO: 89 - protein, 212 aa, Artificial
  Synthetic polypeptide/peptide
ACAGTGCAGGGGAAAGAATAGTAGACATAATAGCAACAGACATACAAACTAAAGAATTACAAAAACAAATTACAAAAATTCAAAATTTTCCGATCACGAGACTAGCCTCGAGAAGCTTGATCGATGGCTCCGGTGCCCGTCAGTGGGCAGAGCGCACATCGCCCACAGTCCCCGAGAAGTTGGGGGGAGGGGTCGGCAATTGAACCGGTGCC